European Patent Specification EP 3 546 575 B1, published July 17, 2024. Title: Genome editing method. Applicant: Osaka University. The sequence listing filed with the application follows.

SEQUENCE LISTING (17 sequences)

SEQ ID NO: 1 - DNA, 268 bp, Mus musculus
acagtggactgaaggagccacggagtccagggactcttcctttctctttcattctcaggatgatagatgagctccacctgcccaagttctccatctccaccgactacagcctggaggatgtcctttcaaagctgggcatcagggaagtcttctccacacaggctgacctgtctgcaatcacaggaaccaaggatctgagagtctctcaggtaagacaaagaagcacttggtggttcagcttgtgccctgaacgtggatggtgagggcc

SEQ ID NO: 2 - DNA, 23 bp, Artificial Sequence
  Serpina3a gRNA-1 target strand
gagaagccccagcgtcacagtgg

SEQ ID NO: 3 - DNA, 23 bp, Artificial Sequence
  Serpina3a gRNA-2 target strand
gtggatggtgagggccacgaggg

SEQ ID NO: 4 - DNA, 695 bp, Artificial Sequence
  lssDNA for Serpina3a
gttaataatctgagtgctggtcaagaagtcctggagggaagaagttgaggctgggtgtgctttgtgactgcagtggattggagggggggggcacctgcggtgcagcacagatcggtacccatgtgatctaacaccaagcataggcacttcctcatcatgggttcctgggtgtggttatatccagggagtaaagtagtactgctctctgcaggagtatctgggggttttaagctcccccagcgtgagaaaaactgagaaatataggtcttctcacacgtgtgccaatcccacatgccctcgtataacttcgtatagcatacattatacgaagttatggccctcaccatccacgttcagggcacaagctgaaccaccaagtgcttctttgtcttacctgagagactctcagatccttggttcctgtgattgcagacaggtcagcctgtgtggagaagacttccctgatgcccagctttgaaaggacatcctccaggctgtagtcggtggagatggagaacttgggcaggtggagctcatctatcatcctgagaatgaaagagaaaggaagagtccctggactccgtggctccttcagtccactgtataacttcgtatagcatacattatacgaagttatgacgctggggcttctctacacagagagtcctctaactacagggaagtcctcttcccag

SEQ ID NO: 5 - DNA, 467 bp, Mus musculus
atggtaggttaagttcactttcatctaactgccagaaagctgaatgatactgatgtgcaatttcaacatctttctcttgtctcagaagtaactcatttaacataaattgtttttcacagatcatttgtagcagatcagaagagtataatagccatcaggttttatgcgatggaacacctgagggaccactattacgtaatcctggaaaccatgacaaagccaaaacccccaggctcccatcttcagcagatgtggaattttgtctgagtttgacccagtatgaatctggatcaatggatagaactgccaatttcagctttagaaacacactggaaggtaatatccttgtgttcattaattttgattttttttaatttataatttcttttcagaaattctgggctcagagatgtttataatttaaaattttgtgagttttgaaatgttatgcttcaattatacccatg

SEQ ID NO: 6 - DNA, 23 bp, Artificial Sequence
  Tyr gRNA-1 non-target strand
cctagcatggtaggttaagttca

SEQ ID NO: 7 - DNA, 23 bp, Artificial Sequence
  Tyr gRNA-2 non-target strand
cccatggtgatagtaaacttagc

SEQ ID NO: 8 - DNA, 905 bp, Artificial Sequence
  lssDNA for Tyr
tatatgaaagattgtgaagaacttttaataatatttggtaggtaatttctgtaagtgttgttggaggttatccccaatgtttgctcgtgtatgaatctggggcttgaggggtcttccctcccttcccttcccttcccttcccttcccttcccttcccttcccttcccttcccttcccttcccttcccttcccttcccttccctttccttttctttcctttccttcgcttccctttcccttttatatcactaaatttctggagtatagtgagatactctatgctagctaagtttactatcaataacttcgtatagcatacattatacgaagttatccatgggtataattgaagcataacatttcaaaactcacaagcttcatgtggtcggggtagaattttaaattataaacatctctgagcccagaatttctgaaaagaaattataaattaaaaaaaatcaaaattaatgaacacaaggatattaccttccagtgtgtttctaaagctgaaattggcagttctatccattgatccagattcatactgggtcaaactcagacaaaattccacatctgctgaagatgggagcctgggggttttggctttgtcatggtttccaggattacgtaatagtggtccctcaggtgttccatcgcataaaacctgatggctattatactcttctgatctgctacaaatgatctgtgaaaaacaatttatgttaaatgagttacttctgagacaagagaaagatgttgaaattgcacatcagtatcattcagctttctggcagttagatgaaagtgaacttaacctaccaataacttcgtatagcatacattatacgaagttattgctaggcatttattattattgtggctggcactcgctagtctaatttgtg

SEQ ID NO: 9 - DNA, 662 bp, Mus musculus
ccagtggtcaggttccacaagcagtttcttcaaaggtgcttgatgcctgctgccctgcttgggcatcgtgaggagctgagccatgcctagggtccatgagtcacctgcactaaggacctgacaccccagtgctcagcacccctgttaggctgagggcagagctaagctggaggcctggacctgccctcagctaccttccccacacaggaccgctctgcagtgtgtgtgtgaaccgctttggctgccggcctgtcatgcttgtgggtggcctctttgcgtccctgggaatggtggctgcgtccttctgcagaagcattatccagatctacctcaccacgggggtcatcactggtgagtccggtgggacctgaagacctcagggtgtcaggaaagatgagtgggccatggcacttgtgctcatctgttccaagctttgggggaaagttgaagactcttgggcccctgggctatgtgtagccttccctcccatccacaatagtccccgagagcagtaggtacagccctgctggggtcgagtggctggtgtctgagggcttggacgtcgagacccatttagaagcttgtcatcatctggagcccaagtccaggggatctggggagtggacaaaggtctggggaaacacagggatctaagctgcctt

SEQ ID NO: 10 - DNA, 23 bp, Artificial Sequence
  Mct4 gRNA-1 target strand
ggttgtgccgatactcccagtgg

SEQ ID NO: 11 - DNA, 23 bp, Artificial Sequence
  Mct4 gRNA-2 target strand
ggatctaagctgccttgcttggg

SEQ ID NO: 12 - DNA, 1083 bp, Artificial Sequence
  lssDNA for Mct4
cccgatgggggctggggctgggccgtcctctttggctgttttatcatcacgggtttctcctacgccttccccaaggcggtcagcgtctttttcaaggagcttatgcatgagtttgggattggctacagcgacacggcttggatctcctccatcctgctggctatgctctatggcacaggtgaggtgggggggggggcacagggagcatgggcgaatgggcgaatgggttaaatcttgggggaggtgatcttgccagagagctattggctctgtctcagggggtgggttgtgccgatactcataacttcgtataatgtatgctatacgaagttatccagtggtcaggttccacaagcagtttcttcaaaggtgcttgatgcctgctgccctgcttgggcatcgtgaggagctgagccatgcctagggtccatgagtcacctgcactaaggacctgacaccccagtgctcagcacccctgttaggctgagggcagagctaagctggaggcctggacctgccctcagctaccttccccacacaggaccgctctgcagtgtgtgtgtgaaccgctttggctgccggcctgtcatgcttgtgggtggcctctttgcgtccctgggaatggtggctgcgtccttctgcagaagcattatccagatctacctcaccacgggggtcatcactggtgagtccggtgggacctgaagacctcagggtgtcaggaaagatgagtgggccatggcacttgtgctcatctgttccaagctttgggggaaagttgaagactcttgggcccctgggctatgtgtagccttccctcccatccacaatagtccccgagagcagtaggtacagccctgctggggtcgagtggctggtgtctgagggcttggacgtcgagacccatttagaagcttgtcatcatctggagcccaagtccaggggatctggggagtggacaaaggtctggggaaacacagggatctaagctgccttataacttcgtataatgtatgctatacgaagttatgcttgggaatctgagtcatgccttccctgcaggcttggatctcagagtctcac

SEQ ID NO: 13 - DNA, 210 bp, Rattus norvegicus
cacaggacaccaaccattttctgtctctccacgtaggtcccttcactgatgttgtcactaccaacctaaagctgggcaacccgacagaccggaacgtgtgtttcaaagtgaagaccacagcgccgcgcaggtactgcgtgcggcccaacagtggggtcattgatgccggggcctctctcaatgtgtctggtaagtcccaaaccgagaggt

SEQ ID NO: 14 - DNA, 23 bp, Artificial Sequence
  Vapb gRNA-1 target strand
tgagctcctactttcctcacagg

SEQ ID NO: 15 - DNA, 23 bp, Artificial Sequence
  Vapb gRNA-2 target strand
gtcccaaaccgagaggtcatggg

SEQ ID NO: 16 - DNA, 210 bp, Artificial Sequence
  mutated genome editing region
cacaggacaccaaccattttctgtctctccacgtaggtcccttcactgatgttgtcactaccaacctaaagctgggcaacccgacagaccggaacgtgtgtttcaaagtgaagaccacagcgccgcgcaggtactgcgtgcggtccaacagtggggtcattgatgccggggcctctctcaatgtgtctggtaagtcccaaaccgagaggt

SEQ ID NO: 17 - DNA, 585 bp, Artificial Sequence
  lssDNA for Vapb
cccttgcagacacactggtaggagttttcctgtctacagaatcgcatcctcccagagtctacctgacacctgacactctgcccttcatagtcactggggatccatgcctggtcctttgtacagtttctgccggattccactgtggttctgtggaagcaagtgttgatcatgagtgactgttgtaggattcattgtgtctaggtcctttcacttctcagaggtctcctgtcttcctgagctcctactttcctataacttcgtataatgtatgctatacgaagttatcacaggacaccaaccattttctgtctctccacgtaggtcccttcactgatgttgtcactaccaacctaaagctgggcaacccgacagaccggaacgtgtgtttcaaagtgaagaccacagcgccgcgcaggtactgcgtgcggtccaacagtggggtcattgatgccggggcctctctcaatgtgtctggtaagtcccaaaccgagaggtataacttcgtataatgtatgctatacgaagttatcatgggtggggtccagaagccccagagccatcgagcctggtcagaatgggtagtcc